European Patent Application EP 4 534 658 A1, published April 9, 2025. Title: Novel variant of ABC transporter permease and method for producing 5'-inosinic acid using the same. Applicant: DAESANG CORPORATION. The sequence listing filed with the application follows.

SEQUENCE LISTING (9 sequences)

SEQ ID NO: 1 - DNA, 687 bp, synthetic construct
  source 1..687: mol_type = other DNA
atgaacgccatgtgggatcagctattatctggcttatggccagcattttggctaaccatccaactgactttttggtcggcgattggttcgacaatcctcggaaccatcctcaccgccatgcgcgtctccccggttgcgattttgtgcaccatatccacgttctatatttctgtggttcgcaatactcccctgacgctcatcgtcctattctgttcctttggtctctatcagaacctgggaatggctctagctagccgcgaatccgctagtttcctggtggataataacttccgcctcgctatagtgggctttatcctctacacctcagcctttgtcgccgagtccttgcgttctggtatcaacaccgtcgactttggccaagcagaagcagcccgctcgctgggattgagcttttctgacatgttcagaaagattgtcttcccacaagcagttcgcgcggctatcgtgcctttgggaaatacgcttatcgcgttgaccaagaacatcaccattgcttcaacaatcggtgtcgcagaagcgtccctgttaatgaagtcgacaatcgaaaaccacgcgaatcagctcttcatcatcttcttcgtcttcgcgcttggtttcatcatcctcaccctgcccatgggccttgggttaggcaaactttctgaaagaatggcggtgaagaagtaa

SEQ ID NO: 2 - protein, 228 aa, synthetic construct
MNAMWDQLLSGLWPAFWLTIQLTFWSAIGSTILGTILTAMRVSPVAILCTISTFYISVVRNTPLTLIVLFCSFGLYQNLGMALASRESASFLVDNNFRLAIVGFILYTSAFVAESLRSGINTVDFGQAEAARSLGLSFSDMFRKIVFPQAVRAAIVPLGNTLIALTKNITIASTIGVAEASLLMKSTIENHANQLFIIFFVFALGFIILTLPMGLGLGKLSERMAVKK

SEQ ID NO: 3 - DNA, 687 bp, Corynebacterium stationis
  source 1..687: mol_type = genomic DNA
atgaacgccatgtgggatcagctattacctggcttatggccagcattttggctaaccatccaactgactttttggtcggcgattggttcgacaatcctcggaaccatcctcaccgccatgcgcgtctccccggttgcgattttgcgcaccatatccacgttctatatttctgtggttcgcaatactcccctgacgctcatcgtcctattctgttcctttggtctctatcagaacctgggaatggctctagctagccgcgaatccgctagtttcctggtggataataacttccgcctcgctatagtgggctttatcctctacacctcagcctttgtcgccgagtccttgcgttctggtatcaacaccgtcgactttggccaagcagaagcagcccgctcgctgggattgagcttttctgacatgttcagaaagattgtcttcccacaagcagttcgcgcggctatcgtgcctttgggaaatacgcttatcgcgttgaccaagaacaccaccattgcttcaacaatcggtgtcgcagaagcgtccctgttaatgaagtcgacaatcgaaaaccacgcgaatcagctcttcatcatcttcttcgtcttcgcgcttggtttcatcatcctcaccctgcccatgggccttgggttaggcaaactttctgaaagaatggcggtgaagaagtaa

SEQ ID NO: 4 - protein, 228 aa, Corynebacterium stationis
MNAMWDQLLPGLWPAFWLTIQLTFWSAIGSTILGTILTAMRVSPVAILRTISTFYISVVRNTPLTLIVLFCSFGLYQNLGMALASRESASFLVDNNFRLAIVGFILYTSAFVAESLRSGINTVDFGQAEAARSLGLSFSDMFRKIVFPQAVRAAIVPLGNTLIALTKNTTIASTIGVAEASLLMKSTIENHANQLFIIFFVFALGFIILTLPMGLGLGKLSERMAVKK

SEQ ID NO: 5 - DNA, 5719 bp, synthetic construct
  source 1..5719: mol_type = other DNA
tgccgcaagcactcagggcgcaagggctgctaaaggaagcggaacacgtagaaagccagtccgcagaaacggtgctgaccccggatgaatgtcagctactgggctatctggacaagggaaaacgcaagcgcaaagagaaagcaggtagcttgcagtgggcttacatggcgatagctagactgggcggttttatggacagcaagcgaaccggaattgccagctggggcgccctctggtaaggttgggaagccctgcaaagtaaactggatggctttcttgccgccaaggatctgatggcgcaggggatcaagatctgatcaagagacaggatgaggatcgtttcgcatgattgaacaagatggattgcacgcaggttctccggccgcttgggtggagaggctattcggctatgactgggcacaacagacaatcggctgctctgatgccgccgtgttccggctgtcagcgcaggggcgcccggttctttttgtcaagaccgacctgtccggtgccctgaatgaactccaagacgaggcagcgcggctatcgtggctggccacgacgggcgttccttgcgcagctgtgctcgacgttgtcactgaagcgggaagggactggctgctattgggcgaagtgccggggcaggatctcctgtcatctcaccttgctcctgccgagaaagtatccatcatggctgatgcaatgcggcggctgcatacgcttgatccggctacctgcccattcgaccaccaagcgaaacatcgcatcgagcgagcacgtactcggatggaagccggtcttgtcgatcaggatgatctggacgaagagcatcaggggctcgcgccagccgaactgttcgccaggctcaaggcgcggatgcccgacggcgaggatctcgtcgtgacccatggcgatgcctgcttgccgaatatcatggtggaaaatggccgcttttctggattcatcgactgtggccggctgggtgtggcggaccgctatcaggacatagcgttggctacccgtgatattgctgaagagcttggcggcgaatgggctgaccgcttcctcgtgctttacggtatcgccgctcccgattcgcagcgcatcgccttctatcgccttcttgacgagttcttctgagcgggactctggggttcgctagaggatcgatcctttttaacccatcacatatacctgccgttcactattatttagtgaaatgagatattatgatattttctgaattgtgattaaaaaggcaactttatgcccatgcaacagaaactataaaaaatacagagaatgaaaagaaacagatagattttttagttctttaggcccgtagtctgcaaatccttttatgattttctatcaaacaaaagaggaaaatagaccagttgcaatccaaacgagagtctaatagaatgaggtcgaaaagtaaatcgcgcgggtttgttactgataaagcaggcaagacctaaaatgtgtaaagggcaaagtgtatactttggcgtcaccccttacatattttaggtctttttttattgtgcgtaactaacttgccatcttcaaacaggagggctggaagaagcagaccgctaacacagtacataaaaaaggagacatgaacgatgaacatcaaaaagtttgcaaaacaagcaacagtattaacctttactaccgcactgctggcaggaggcgcaactcaagcgtttgcgaaagaaacgaaccaaaagccatataaggaaacatacggcatttcccatattacacgccatgatatgctgcaaatccctgaacagcaaaaaaatgaaaaatatcaagtttctgaatttgattcgtccacaattaaaaatatctcttctgcaaaaggcctggacgtttgggacagctggccattacaaaacgctgacggcactgtcgcaaactatcacggctaccacatcgtctttgcattagccggagatcctaaaaatgcggatgacacatcgatttacatgttctatcaaaaagtcggcgaaacttctattgacagctggaaaaacgctggccgcgtctttaaagacagcgacaaattcgatgcaaatgattctatcctaaaagaccaaacacaagaatggtcaggttcagccacatttacatctgacggaaaaatccgtttattctacactgatttctccggtaaacattacggcaaacaaacactgacaactgcacaagttaacgtatcagcatcagacagctctttgaacatcaacggtgtagaggattataaatcaatctttgacggtgacggaaaaacgtatcaaaatgtacagcagttcatcgatgaaggcaactacagctcaggcgacaaccatacgctgagagatcctcactacgtagaagataaaggccacaaatacttagtatttgaagcaaacactggaactgaagatggctaccaaggcgaagaatctttatttaacaaagcatactatggcaaaagcacatcattcttccgtcaagaaagtcaaaaacttctgcaaagcgataaaaaacgcacggctgagttagcaaacggcgctctcggtatgattgagctaaacgatgattacacactgaaaaaagtgatgaaaccgctgattgcatctaacacagtaacagatgaaattgaacgcgcgaacgtctttaaaatgaacggcaaatggtacctgttcactgactcccgcggatcaaaaatgacgattgacggcattacgtctaacgatatttacatgcttggttatgtttctaattctttaactggcccatacaagccgctgaacaaaactggccttgtgttaaaaatggatcttgatcctaacgatgtaacctttacttactcacacttcgctgtacctcaagcgaaaggaaacaatgtcgtgattacaagctatatgacaaacagaggattctacgcagacaaacaatcaacgtttgcgccgagcttcctgctgaacatcaaaggcaagaaaacatctgttgtcaaagacagcatccttgaacaaggacaattaacagttaacaaataaaaacgcaaaagaaaatgccgatgggtaccgagcgaaatgaccgaccaagcgacgcccaacctgccatcacgagatttcgattccaccgccgccttctatgaaaggttgggcttcggaatcgttttccgggacgccctcgcggacgtgctcatagtccacgacgcccgtgattttgtagccctggccgacggccagcaggtaggccgacaggctcatgccggccgccgccgccttttcctcaatcgctcttcgttcgtctggaaggcagtacaccttgataggtgggctgcccttcctggttggcttggtttcatcagccatccgcttgccctcatctgttacgccggcggtagccggccagcctcgcagagcaggattcccgttgagcaccgccaggtgcgaataagggacagtgaagaaggaacacccgctcgcgggtgggcctacttcacctatcctgcccggctgacgccgttggatacaccaaggaaagtctacacgaaccctttggcaaaatcctgtatatcgtgcgaaaaaggatggatataccgaaaaaatcgctataatgaccccgaagcagggttatgcagcggaaaagcgctgcttccctgctgttttgtggaatatctaccgactggaaacaggcaaatgcaggaaattactgaactgaggggacaggcgagagacgatgccaaagagctcctgaaaatctcgataactcaaaaaatacgcccggtagtgatcttatttcattatggtgaaagttggaacctcttacgtgccgatcaacgtctcattttcgccaaaagttggcccagggcttcccggtatcaacagggacaccaggatttatttattctgcgaagtgatcttccgtcacaggtatttattcggcgcaaagtgcgtcgggtgatgctgccaacttactgatttagtgtatgatggtgtttttgaggtgctccagtggcttctgtttctatcagctcctgaaaatctcgataactcaaaaaatacgcccggtagtgatcttatttcattatggtgaaagttggaacctcttacgtgccgatcaacgtctcattttcgccaaaagttggcccagggcttcccggtatcaacagggacaccaggatttatttattctgcgaagtgatcttccgtcacaggtatttattcggcgcaaagtgcgtcgggtgatgctgccaacttactgatttagtgtatgatggtgtttttgaggtgctccagtggcttctgtttctatcagggctggatgatcctccagcgcggggatctcatgctggagttcttcgcccaccccaaaaggatctaggtgaagatcctttttgataatctcatgaccaaaatcccttaacgtgagttttcgttccactgagcgtcagaccccgtagaaaagatcaaaggatcttcttgagatcctttttttctgcgcgtaatctgctgcttgcaaacaaaaaaaccaccgctaccagcggtggtttgtttgccggatcaagagctaccaactctttttccgaaggtaactggcttcagcagagcgcagataccaaatactgttcttctagtgtagccgtagttaggccaccacttcaagaactctgtagcaccgcctacatacctcgctctgctaatcctgttaccagtggctgctgccagtggcgataagtcgtgtcttaccgggttggactcaagacgatagttaccggataaggcgcagcggtcgggctgaacggggggttcgtgcacacagcccagcttggagcgaacgacctacaccgaactgagatacctacagcgtgagctatgagaaagcgccacgcttcccgaagggagaaaggcggacaggtatccggtaagcggcagggtcggaacaggagagcgcacgagggagcttccagggggaaacgcctggtatctttatagtcctgtcgggtttcgccacctctgacttgagcgtcgatttttgtgatgctcgtcaggggggcggagcctatggaaaaacgccagcaacgcggcctttttacggttcctggccttttgctggccttttgctcacatgttctttcctgcgttatcccctgattctgtggataaccgtattaccgcctttgagtgagctgataccgctcgccgcagccgaacgaccgagcgcagcgagtcagtgagcgaggaagcggaagagcgcccaatacgcaaaccgcctctccccgcgcgttggccgattcattaatgcagctggcacgacaggtttcccgactggaaagcgggcagtgagcgcaacgcaattaatgtgagttagctcactcattaggcaccccaggctttacactttatgcttccggctcgtatgttgtgtggaattgtgagcggataacaatttcacacaggaaacagctatgacatgattacgccaagcttgcatgcctgcaggtcgactctagaggatccccgggtaccgagctcgaattcactggccgtcgttttacaacgtcgtgactgggaaaaccctggcgttacccaacttaatcgccttgcagcacatccccctttcgccagctggcgtaatagcgaagaggcccgcaccgatcgcccttcccaacagttgcgcagcctgaatggcgaatggcgataagctagcttcacgc

SEQ ID NO: 6 - DNA, 24 bp, synthetic construct
  source 1..24: mol_type = other DNA
tcagctattatctggcttatggcc

SEQ ID NO: 7 - DNA, 24 bp, synthetic construct
  source 1..24: mol_type = other DNA
cgtggatatggtgcacaaaatcgc

SEQ ID NO: 8 - DNA, 24 bp, synthetic construct
  source 1..24: mol_type = other DNA
gcgattttgtgcaccatatccacg

SEQ ID NO: 9 - DNA, 24 bp, synthetic construct
  source 1..24: mol_type = other DNA
gaagcaatggtgatgttcttggtc